European Patent Application EP 4 796 554 A1, published August 26, 2026. Title: 靶向递送配体. Applicant: 成都新泽利医药科技有限公司. The sequence listing filed with the application follows.

SEQUENCE LISTING (14 sequences)

SEQ ID NO: 1 - RNA, 21 nt, synthetic construct
  source 1..21: mol_type = other RNA; note = sense strand
  modified_base 1: mod_base = OTHER; note = 2'-fluoro
  modified_base 1..2: mod_base = OTHER; note = thiophosphate
  modified_base 2: mod_base = OTHER; note = 2'-O-methyl
  modified_base 3: mod_base = OTHER; note = 2'-fluoro
  modified_base 4: mod_base = OTHER; note = 2'-O-methyl
  modified_base 5: mod_base = OTHER; note = 2'-fluoro
  modified_base 6: mod_base = OTHER; note = 2'-O-methyl
  modified_base 7: mod_base = OTHER; note = 2'-fluoro
  modified_base 8: mod_base = OTHER; note = 2'-O-methyl
  modified_base 9..11: mod_base = OTHER; note = 2'-fluoro
  modified_base 12: mod_base = OTHER; note = 2'-O-methyl
  modified_base 13: mod_base = OTHER; note = 2'-fluoro
  modified_base 14: mod_base = OTHER; note = 2'-O-methyl
  modified_base 15: mod_base = OTHER; note = 2'-fluoro
  modified_base 16: mod_base = OTHER; note = 2'-O-methyl
  modified_base 17: mod_base = OTHER; note = 2'-fluoro
  modified_base 18: mod_base = OTHER; note = 2'-O-methyl
  modified_base 19: mod_base = OTHER; note = 2'-fluoro
  modified_base 20: mod_base = OTHER; note = 2'-O-methyl
  modified_base 21: mod_base = OTHER; note = 2'-fluoro
agcaacatgtgttcaaagtca

SEQ ID NO: 2 - RNA, 23 nt, synthetic construct
  source 1..23: mol_type = other RNA; note = antisense strand
  modified_base 1: mod_base = OTHER; note = 2'-O-methyl
  modified_base 1: mod_base = OTHER; note = thiophosphate
  modified_base 2: mod_base = OTHER; note = 2'-fluoro
  modified_base 3: mod_base = OTHER; note = 2'-O-methyl
  modified_base 4: mod_base = OTHER; note = 2'-fluoro
  modified_base 5: mod_base = OTHER; note = 2'-O-methyl
  modified_base 6: mod_base = OTHER; note = 2'-fluoro
  modified_base 7: mod_base = OTHER; note = 2'-O-methyl
  modified_base 8: mod_base = OTHER; note = 2'-fluoro
  modified_base 9: mod_base = OTHER; note = 2'-O-methyl
  modified_base 10: mod_base = OTHER; note = 2'-fluoro
  modified_base 11..13: mod_base = OTHER; note = 2'-O-methyl
  modified_base 14: mod_base = OTHER; note = 2'-fluoro
  modified_base 15: mod_base = OTHER; note = 2'-O-methyl
  modified_base 16: mod_base = OTHER; note = 2'-fluoro
  modified_base 17: mod_base = OTHER; note = 2'-O-methyl
  modified_base 18: mod_base = OTHER; note = 2'-fluoro
  modified_base 19: mod_base = OTHER; note = 2'-O-methyl
  modified_base 20: mod_base = OTHER; note = 2'-fluoro
  modified_base 21..23: mod_base = OTHER; note = 2'-O-methyl
  modified_base 21..22: mod_base = OTHER; note = thiophosphate
tgactttgaacacatgttgctca

SEQ ID NO: 3 - RNA, 21 nt, synthetic construct
  source 1..21: mol_type = other RNA; note = sense strand
  modified_base 1..6: mod_base = OTHER; note = 2'-O-methyl
  modified_base 1..2: mod_base = OTHER; note = thiophosphate
  modified_base 7: mod_base = OTHER; note = 2'-fluoro
  modified_base 8: mod_base = OTHER; note = 2'-O-methyl
  modified_base 9..11: mod_base = OTHER; note = 2'-fluoro
  modified_base 12..21: mod_base = OTHER; note = 2'-O-methyl
aacagtgttcttgctctataa

SEQ ID NO: 4 - RNA, 23 nt, synthetic construct
  source 1..23: mol_type = other RNA; note = antisense strand
  modified_base 1: mod_base = OTHER; note = 2'-O-methyl
  modified_base 1..2: mod_base = OTHER; note = thiophosphate
  modified_base 2: mod_base = OTHER; note = 2'-fluoro
  modified_base 3..5: mod_base = OTHER; note = 2'-O-methyl
  modified_base 6: mod_base = OTHER; note = 2'-fluoro
  modified_base 7: mod_base = OTHER; note = 2'-O-methyl
  modified_base 8..9: mod_base = OTHER; note = 2'-fluoro
  modified_base 10..13: mod_base = OTHER; note = 2'-O-methyl
  modified_base 14: mod_base = OTHER; note = 2'-fluoro
  modified_base 15: mod_base = OTHER; note = 2'-O-methyl
  modified_base 16: mod_base = OTHER; note = 2'-fluoro
  modified_base 17..23: mod_base = OTHER; note = 2'-O-methyl
  modified_base 21..22: mod_base = OTHER; note = thiophosphate
ttatagagcaagaacactgtttt

SEQ ID NO: 5 - RNA, 21 nt, synthetic construct
  source 1..21: mol_type = other RNA; note = sense strand
  modified_base 1..6: mod_base = OTHER; note = 2'-O-methyl
  modified_base 1..2: mod_base = OTHER; note = thiophosphate
  modified_base 7: mod_base = OTHER; note = 2'-fluoro
  modified_base 8: mod_base = OTHER; note = 2'-O-methyl
  modified_base 9..11: mod_base = OTHER; note = 2'-fluoro
  modified_base 12..21: mod_base = OTHER; note = 2'-O-methyl
aacagtgttcttgctctataa

SEQ ID NO: 6 - RNA, 21 nt, synthetic construct
  source 1..21: mol_type = other RNA; note = sense strand
  modified_base 1..6: mod_base = OTHER; note = 2'-O-methyl
  modified_base 1..2: mod_base = OTHER; note = thiophosphate
  modified_base 7: mod_base = OTHER; note = 2'-fluoro
  modified_base 8: mod_base = OTHER; note = 2'-O-methyl
  modified_base 9: mod_base = OTHER; note = 2'-fluoro
  modified_base 10: mod_base = OTHER; note = 2'-O-methyl
  modified_base 11: mod_base = OTHER; note = T is dT
  modified_base 12..21: mod_base = OTHER; note = 2'-O-methyl
ctagacctgttttgcttttgt

SEQ ID NO: 7 - RNA, 23 nt, synthetic construct
  source 1..23: mol_type = other RNA; note = antisense strand
  modified_base 1: mod_base = OTHER; note = 2'-O-methyl
  modified_base 1..2: mod_base = OTHER; note = thiophosphate
  modified_base 2: mod_base = OTHER; note = 2'-fluoro
  modified_base 3: mod_base = OTHER; note = 2'-O-methyl
  modified_base 4..6: mod_base = OTHER; note = 2'-fluoro
  modified_base 7: mod_base = OTHER; note = 2'-O-methyl
  modified_base 8: mod_base = OTHER; note = 2'-fluoro
  modified_base 9: mod_base = OTHER; note = 2'-O-methyl
  modified_base 10: mod_base = OTHER; note = 2'-fluoro
  modified_base 11: mod_base = OTHER; note = 2'-O-methyl
  modified_base 12: mod_base = OTHER; note = 2'-fluoro
  modified_base 13: mod_base = OTHER; note = 2'-O-methyl
  modified_base 14: mod_base = OTHER; note = 2'-fluoro
  modified_base 15: mod_base = OTHER; note = 2'-O-methyl
  modified_base 16: mod_base = OTHER; note = 2'-fluoro
  modified_base 17: mod_base = OTHER; note = 2'-O-methyl
  modified_base 18: mod_base = OTHER; note = 2'-fluoro
  modified_base 19..23: mod_base = OTHER; note = 2'-O-methyl
  modified_base 21..22: mod_base = OTHER; note = thiophosphate
acaaaagcaaaacaggtctagaa

SEQ ID NO: 8 - RNA, 21 nt, synthetic construct
  source 1..21: mol_type = other RNA; note = sense strand
  modified_base 1..6: mod_base = OTHER; note = 2'-O-methyl
  modified_base 1..2: mod_base = OTHER; note = thiophosphate
  modified_base 7: mod_base = OTHER; note = 2'-fluoro
  modified_base 8: mod_base = OTHER; note = 2'-O-methyl
  modified_base 9: mod_base = OTHER; note = 2'-fluoro
  modified_base 10: mod_base = OTHER; note = 2'-O-methyl
  modified_base 11: mod_base = OTHER; note = T is dT
  modified_base 12..21: mod_base = OTHER; note = 2'-O-methyl
ctagacctgttttgcttttgt

SEQ ID NO: 9 - DNA, 21 bp, synthetic construct
  source 1..21: mol_type = other DNA; note = primer
ctgctgtagacgtggctgtaa

SEQ ID NO: 10 - DNA, 22 bp, synthetic construct
  source 1..22: mol_type = other DNA; note = primer
cttccagtacgatttggtgtcc

SEQ ID NO: 11 - DNA, 26 bp, synthetic construct
  source 1..26: mol_type = other DNA; note = primer
aagacctctgagggatcctgggagcc

SEQ ID NO: 12 - DNA, 20 bp, synthetic construct
  source 1..20: mol_type = other DNA; note = primer
ctgcaccaccaactgcttag

SEQ ID NO: 13 - DNA, 20 bp, synthetic construct
  source 1..20: mol_type = other DNA; note = primer
ggatgcagggatgatgttct

SEQ ID NO: 14 - DNA, 29 bp, synthetic construct
  source 1..29: mol_type = other DNA; note = primer
tggccaaggtcatccatgacaactttggc